European Patent Application EP 4 400 577 A1, published July 17, 2024. Title: NOVEL BACTERIA FOR MASS PRODUCTION OF PROPIONIC ACID PRECURSORS. Applicant: National Agriculture and Food Research Organization. The sequence listing filed with the application follows.

SEQUENCE LISTING (13 sequences)

SEQ ID NO: 1 - DNA, 1492 bp, Prevotella sp.
agagtttgatcctggctcaggatgaacgctagctacaggcttaacacatgcaagtcgaggggtaacgacagcgaaagcttgcttttgctgggcgacgaccggcgaatgggtgagtaacgcgtatccaacctgccgcaaagtagggcacagccttgcgaaagtaagattaatgccctatgtgctgtgatgaggacatctgaattgcagtaaaggtttaccgctttgcgatggggatgcgtctgattaggttgttggcggggtaacggcccaccaagcccgcgatcagtaggggttctgagaggaaggtcccccacattggaactgagacacggtccaaactcctacgggaggcagcagtgaggaatattggtcaatgggcgagagcctgaaccagccaagtagcgtgcgggacgaaggccctatgggttgtaaaccgcttttacggggggataaagtgagtgacgtgtcattcattgcaggtaccccgcgaataaggaccggctaattccgtgccagcagccgcggtaatacggaaggtccgggcgttatccggatttattgggtttaaagggagcacaggccggctgtcaagcgtgttgtgaaatgtaggcgctcaacgcctgacttgcagcgcgaactgacggtcttgagtgcgcgcaacgttggcggaatttgtcgtgtagcggtgaaatgcttagatatgacgaagaactccgattgcgaaggcagctgacgggagcgttactgacgcttaagctcgaaagcgcgggtatcgaacaggattagataccctggtagtccgcgcggtaaacgatggatgcccgctgtttgcgtctaacgtaagcggccaagtgaaaacgttaagcatcccacctggggagtacgccggcaacggtgaaactcaaaggaattgacgggggcccgcacaagcggaggaacatgtggtttaattcgatgatacgcgaggaaccttacccgggcttgaattgctgaggaaagatccagagatggtgatgcccttcggggcctcggtgaaggtgctgcatggttgccgtcagctcgtgccgtgaggtgtcggcttaagtgccataacgagcgcaacccctctcttcagttgccatcaggctatgctgggcactctggagacactgccaccgcaaggtgtgaggaaggtggggatgacgtcaaatcagcacggcccttacgtccggggctacacacgtgttacaatggggggcacagagagcggggtgcgcgcaagcttgcccaaatccttaaatccccccacagttcggactggggtctgcaacccgaccccacgaagctggattcgctagtaatcgcgcatcagccatggcgcggtgaatacgttcccgggccttgtacacaccgcccgtcaagccatgaaagccgggggtgcctgaagtccgtgaccgcaagggacggcctagggcaaaactggtaattggggctaagtcgtaacaaggtaacc

SEQ ID NO: 2 - DNA, 1492 bp, Prevotella sp.
agagtttgatcatggctcaggatgaacgctagctacaggcttaacacatgcaagtcgaggggtaacgacagcgaaagcttgcttttgctgggcgacgaccggcgaatgggtgagtaacgcgtatccaacctgccgcaaagtagggcacagccttgcgaaagtaagattaatgccctatgtgctgtgatgatgacatcagaattgcagtaaaggttcaccgctttgcgatggggatgcgtctgattaggttgtcggcggggtaacggcccacctagcccgcgatcagtaggggttctgagaggaaggtcccccacattggaactgagacacggtccaaactcctacgggaggcagcagtgaggaatattggtcaatgggcgagagcctgaaccagccaagtagcgtgcgggacgaaggccctatgggttgtaaaccgcttttacggggggataaagtgagtgacgtgtcattcattgcaggtaccccgcgaataaggaccggctaattccgtgccagcagccgcggtaatacggaaggtccgggcgttatccggatttattgggtttaaagggagcacaggccggctgtcaagcgtgttgtgaaatgtaggcgctcaacgcctgacttgcagcgcgaactgacggtcttgagtgcgcgcaacgttggcggaatttgtcgtgtagcggtgaaatgcttagatatgacgaagaactccgattgcgaaggcagctgacgggagcgttactgacgcttaagctcgaaagcgcgggtatcgaacaggattagataccctggtagtccgcgcggtaaacgatggatgcccgctgtttgcgtctaacgtaagcggccaagtgaaaacgttaagcatcccacctggggagtacgccggcaacggtgaaactcaaaggaattgacgggggcccgcacaagcggaggaacatgtggtttaattcgatgatacgcgaggaaccttacccgggcttgaattgctgaggaaagatccagagatggtgatgcccttcggggcctcagtgaaggtgctgcatggttgtcgtcagctcgtgccgtgaggtgtcggcttaagtgccataacgagcgcaacccctctcttcagttgccatcaggtcaagctgggcactctggagacactgccaccgcaaggtgtgaggaaggtggggatgacgtcaaatcagcacggcccttacgtccggggctacacacgtgttacaatggggggcacagagagcggggtgcgcgcaagcttgcccaaatccttaaatccccccacagttcggactggggtctgcaacccgaccccacgaagctggattcgctagtaatcgcgcatcagccatggcgcggtgaatacgttcccgggccttgtacacaccgcccgtcaagccatgaaagccgggggtgcctgaagtccgtgaccgcaagggacggcctagggcaaaactggcaattggggctaagtcgtaacaaggtagcc

SEQ ID NO: 3 - DNA, 1492 bp, Prevotella sp.
agagtttgatcctggctcaggatgaacgctagctacaggcttaacacatgcaagtcgaggggtaacgacagcgaaagcttgcttttgctgggcgacgaccggcgaatgggtgagtaacgcgtatccaacctgccgcaaagtagggcacagccttgcgaaagtaggattaatgccctatgtgctgtgatgatgacatcagaattgcagtaaaggttcaccgctttgcgatggggatgcgtctgattaggttgttggcggggtaacggcccaccaagcccgcgatcagtaggggttctgagaggaaggtcccccacattggaactgagacacggtccaaactcctacgggaggcagcagtgaggaatattggtcaatgggcgagagcctgaaccagccaagtagcgtgcgggacgaaggccctatgggttgtaaaccgcttttacggggggataaagtgagtgacgtgtcattcattgcaggtaccccgcgaataaggaccggctaattccgtgccagcagccgcggtaatacggaaggtccgggcgttatccggatttattgggtttaaagggagcacaggccggctgtcaagcgtgttgtgaaatgtaggcgctcaacgcctgacttgcagcgcgaactgacggtcttgagtgcgcgcaacgttggcggaatttgtcgtgtagcggtgaaatgcttagatatgacgaagaactccgattgcgaaggcagctgacgggagcgttactgacgcttaagctcgaaagcgcgggtatcgaacaggattagataccctggtagtccgcgcggtaaacgatggatgcccgctgtttgcgtctaacgtaagcggccaagtgaaaacgttaggcatcccacctggggagtacgccggcaacggtgaaactcaaaggaattgacgggggcccgcacaagcggaggaacatgtggtttaattcgatgatacgcgaggaaccttacccgggcttgaattgctgaggaaagatccagagatggtgatgcccttcggggcctcagtgaaggtgctgcatggttgtcgtcagctcgtgccgtgaggtgtcggcttaagtgccataacgagcgcaacccctctcttcagttgccatcaggctatgctgggcactctggagacactgccaccgcaaggtgtgaggaaggtggggatgacgtcaaatcagcacggcccttacgtccggggctacacacgtgttacaatggggggcacagagagcggggtgcgcgcaagcttgcccaaatccttaaatccccccacagttcggactggggtctgcaacccgaccccacgaagctggattcgctagtaatcgcgcatcagccatggcgcggtgaatacgttcccgggccttgtacacaccgcccgtcaagccatgaaagccgggggtgcctgaagtccgtgaccgcaagggacggcctagggcaaaactggtaattggggctaagtcgtaacaaggtaacc

SEQ ID NO: 4 - DNA, 1492 bp, Prevotella sp.
agagtttgatcctggctcaggatgaacgctagctacaggcttaacacatgcaagtcgaggggtaacgacagcgaaagcttgcttttgctgggcgacgaccggcgaatgggtgagtaacgcgtatccaacctgccgcaaagtagggcacagccttgcgaaagtaagattaatgccctatgtgctgtgatgatgacatcagaattgcagtaaaggttcaccgctttgcgatggggatgcgtctgattaggttgttggcggggtaacggcccaccaagcccgcgatcagtaggggttctgagaggaaggtcccccacattggaactgagacacggtccaaactcctacgggaggcagcagtgaggaatattggtcaatgggcgagagcctgaaccagccaagtagcgtgcgggacgaaggccctatgggttgtaaaccgcttttacggggggataaagtgagtgacgtgtcattcattgcaggtaccccgcgaataaggaccggctaattccgtgccagcagccgcggtaatacggaaggtccgggcgttatccggatttattgggtttaaagggagcacaggccggctgtcaagcgtgttgtgaaatgtaggcgctcaacgcctgacttgcagcgcgaactgacggtcttgagtgcgcgcaacgttggcggaatttgtcgtgtagcggtgaaatgcttagatatgacgaagaactccgattgcgaaggcagctgacgggagcgttactgacgcttaagctcgaaagcgcgggtatcgaacaggattagataccctggtagtccgcgcggtaaacgatggatgcccgctgtttgcgtctaacgtaagcggccaagtgaaaacgttaagcatcccacctggggagtacgccggcaacggtgaaactcaaaggaattgacgggggcccgcacaagcggaggaacatgtggtttaattcgatgatacgcgaggaaccttacccgggcttgaattgctgaggaaagatccagagatggtgatgcctttcggggcctcagtgaaggtgctgcatggttgtcgtcagctcgtgccgtgaggtgtcggcttaagtgccataacgagcgcaacccctctcttcagttgccatcaggtcaagctgggcactctggagacactgccaccgcaaggtgtgaggaaggtggggatgacgtcaaatcagcacggcccttacgtccggggctacacacgtgttacaatggggggcacagagagcggggtgcgcgcaagcttgcccaaatccttaaatccccccacagttcggactggggtctgcaacccgaccccacgaagctggattcgctagtaatcgcgcatcagccatggcgcggtgaatacgttcccgggccttgtacacaccgcccgtcaagccatgaaagccgggggtgcctgaagtccgtgaccgcaagggacggcctagggcaaaactggtaattggggctaagtcgtaacaaggtaacc

SEQ ID NO: 5 - DNA, 1492 bp, Prevotella sp.
agagtttgatcatggctcaggatgaacgctagctacaggcttaacacatgcaagtcgaggggtaacgacagcgaaagcttgcttttgctgggcgacgaccggcgaatgggtgagtagcgcgtatccaacctgccgcaaagtagggcacagccttgcgaaagtaagattaatgccctatgtgctgtgatgaggacatctgaattgcagtaaaggtttaccgctttgcgatggggatgcgtctgattaggttgttggcggggtaacggcccaccaagcccgcgatcagtaggggttctgagaggaaggtcccccacattggaactgagacacggtccaaactcctacgggaggcagcagtgaggaatattggtcaatgggcgagagcctgaaccagccaagtagcgtgcgggacgaaggccctatgggttgtaaaccgcttttacggggggataaagtgagtgacgtgtcattcattgcaggtaccccgcgaataaggaccggctaattccgtgccagcagccgcggtaatacggaaggtccgggcgttatccggatttattgggtttaaagggagcacaggccggctgtcaagcgtgttgtgaaatgtaggcgctcaacgcctgacttgcagcgcgaactgacggtcttgagtgcgcgcaacgttggcggaatttgtcgtgtagcggtgaaatgcttagatatgacgaagaactccgattgcgaaggcagctgacgggagcgttactgacgcttaagctcgaaagcgcgggtatcgaacaggattagataccctggtagtccgcgcggtaaacgatggatgcccgctgtttgcgtctaacgtaagcggccaagtgaaaacgttaagcatcccacctggggagtacgccggcaacggtgaaactcaaaggaattgacgggggcccgcacaagcggaggaacatgtggtttaattcgatgatacgcgaggaaccttacccgggcttgaattgctgaggaaagatccagagatggtgatgcccttcggggcctcagtgaaggtgctgcatggttgtcgtcagctcgtgccgtgaggtgtcggcttaagtgccataacgagcgcaacccctctcttcagttgccatcaggctatgctgggcactctggagacactgccaccgcaaggtgtgaggaaggtggggatgacgtcaaatcagcacggcccttacgtccggggctacacacgtgttacaatggggggcgcagagagcggggtgcgcgcaagcttgcccaaatccttaaatccccccacagttcggactggggtctgcaacccgaccccacgaagctggattcgctagtaatcgcgcatcagccatggcgcggtgaatacgttcccgggccttgtacacaccgcccgtcaagccatgaaagccgggggtgcctgaagtccgtgaccgcaagggacggcctagggcaaaactggtaattggggctaagtcgtaacaaggtaacc

SEQ ID NO: 6 - DNA, 1492 bp, Prevotella sp.
agagtttgatcatggctcaggatgaacgctagctacagacttaacacatgcaagtcgaggggtaacgacagcgaaagcttgcttttgctgggcgacgaccggcgaatgggtgagtaacgcgtatccaacctgccgcaaagtagggcacagccttgcgaaagtaagattaatgccctatgtgctgtgatgacgacatcagaattgcagtaaaggttcaccgctttgcgatggggatgcgtctgattaggttgttggcggggtaacggcccaccaagcccgcgatcagtaggggttctgagaggaaggtcccccacattggaactgagacacggtccaaactcctacgggaggcagcagtgaggaatattggtcaatgggcgagagcctgaaccagccaagtagcgtgcgggacgaaggccctatgggttgtaaaccgcttttacggggggataaagtgagtgacgtgtcattcattgcaggtaccccgcgaataaggaccggctaattccgtgccagcagccgcggtaatacggaaggtccgggcgttatccggatttattgggtttaaagggagcacaggccggctgtcaagcgtgttgtgaaatgtaggcgctcaacgcctgacttgcagcgcgaactgacggtcttgagtgcgcgcaacgttggcggaatttgtcgtgtagcggtgaaatgcttagatatgacgaagaactccgattgcgaaggcagctgacgggagcgttactgacgcttaagctcgaaagcgcgggtatcgaacaggattagataccctggtagtccgcgcggtaaacgatggatgcccgctgtttgcgtctaacgtaagcggccaagtgaaaacgttaagcatcccacctggggagtacgccggcaacggtgaaactcaaaggaattgacgggggcccgcacaagcggaggaacatgtggtttaattcgatgatacgcgaggaaccttacccgggcttgaattgctgaggaaagatccagagatggtgatgcccttcggggcctcagtgaaggtgctgcatggttgtcgtcagctcgtgccgtgaggtgtcggcttaagtgccataacgagcgcaacccctctcttcagttgccatcaggtcaagctgggcactctggagacactgccaccgcaaggtgtgaggaaggtggggatgacgtcaaatcagcacggcccttacgtccggggctacacacgtgttacaatggggggcacagagagcggggtgcgcgcaagcttgcccaaatccttaaatccccccacagttcggactggggtctgcaacccgaccccacgaagctggattcgctagtaatcgcgcatcagccatggcgcggtgaatacgttcccgggccttgtacacaccgcccgtcaagccatgaaagccgggggtgcctgaagtccgtgaccgcaagggacggcctagggcaaaactggtaattggggctaagtcgtaacaaggtaacc

SEQ ID NO: 7 - DNA, 1456 bp, Prevotella sp.
agagtttgatcatggctcaggatgaacgctagctacaggcttaacacatgcaagtcgaggggtaacgacagcgaaagcttgcttttgctgggcgacgaccggcgaatgggtgagtaacgcgtatccaacctgccgcaaagtagggcacagccttgcgaaagtaagattaatgccctatgtgctgtgatgatgacatcagaattgcagtaaaggttcaccgctttgcgatggggatgcgtctgattaggttgttggcggggtaacggcccaccaagcccgcgatcagtaggggttctgagaggaaggtcccccacattggaactgagacacggtccaaactcctacgggaggcagcagtgaggaatattggtcaatgggcgagagcctgaaccagccaagtagcgtgcgggacgaaggccctatgggttgtaaaccgcttttacggggggataaagtgagtgacgtgtcattcattgcaggtaccccgcgaataaggaccggctaattccgtgccagcagccgcggtaatacggaaggtccgggcgttatccggatttattgggtttaaagggagcacaggccggctgtcaagcgtgttgtgaaatgtgggcgctcaacgcctgacttgcagcgcgaactgacggtcttgagtgcgcgcaacgttggcggaatttgtcgtgtagcggtgaaatgcttagatatgacgaagaactccgattgcgaaggcagctgacgggagcgttactgacgcttaagctcgaaagcgcgggtatcgaacaggatgcccgctgtttgcgtctaacgtaagcggccaagtgaaaacgttaagcatcccacctggggagtacgccggcaacggtgaaactcaaaggaattgacgggggcccgcacaagcggaggaacatgtggtttaattcgatgatacgcgaggaaccttacccgggcttgaattgctgaggaaagatccagagatggtgatgcccttcggggcctcagtgaaggtgctgcatggttgtcgtcagctcgtgccgtgaggtgtcggcttaagtgccataacgagcgcaacccctctcttcagttgccatcaggctatgctgggcactctggagacactgccaccgcaaggtgtgaggaaggtggggatgacgtcaaatcagcacggcccttacgtccggggctacacacgtgttacaatggggggcacagagagccgggtgcgcgcaagcttgcccaaatccttaaatccccccacagttcggactggggtctgcaacccgaccccacgaagctggattcgctagtaatcgcgcatcagccatggcgcggtgaatacgttcccgggccttgtacacaccgcccgtcaagccatgaaagccgggggtgcctgaagtccgtgaccgcaagggacggcctagggcaaaactggtaattggggctaagtcgtaacaaggtaacc

SEQ ID NO: 8 - DNA, 1456 bp, Prevotella sp.
agagtttgatcctggctcaggatgaacgctagctacaggcttaacacatgcaagtcgaggggtaacgacagcgaaagcttgcttttgctgggcgacgaccggcgaatgggtgagtaacgcgtatccaacctgccgcaaagtagggcacagccttgcgaaagtaagattaatgccctatgtgctgtgatgatgacatcagaattgcagtaaaggttcaccgctttgcgatggggatgcgtctgattaggttgttggcggggtaacggcccaccaagcccgcgatcagtaggggttctgagaggaaggtcccccacattggaactgagacacggtccaaactcctacgggaggcagcagtgaggtatattggtcaatgggcgagagcctgaaccagccaagtagcgtgcgggacgaaggccctatgggttgtaaaccgcttttacggggggataaagtgagtgacgtgtcattcattgcaggtaccccgcgaataaggaccggctaattccgtgccagcagccgcggtaatacggaaggtccgggcgttatccggatttattgggtttaaagggagcacaggccggctgtcaagcgtgttgtgaaatgtaggcgctcaacgcctgacttgcagcgcgaactgacggtcttgagtgcgcgcaacgttggcggaatttgtcgtgtagcggtgaaatgcttagatatgacgaagaactccgattgcgaaggcagctgacgggagcgttactgacgcttaagctcgaaagcgcgggtatcgaacaggatgcccgctgtttgcgtctaacgtaagcggccaagtgaaaacgttaagcatcccacctggggagtacgccggcaacggtgaaactcaaaggaattgacgggggcccgcacaagcggaggaacatgtggtttaattcgatgatacgcgaggaaccttacccgggcttgaattgctgaggaaagatccagagatggtgatgcccttcggggcctcagtgaaggtgctgcatggttgtcgtcagctcgtgccgtgaggtgtcggcttaagtgccataacgagcgcaacccctctcttcagttgccatcaggctatgctgggcactctggagacactgccaccgcaaggtgtgaggaaggtggggatgacgtcaaatcagcacggcccttacgtccggggctacacacgtgttacaatggggggcacagagagccgggtgcgcgcaagcttgcccaaatccttaaatccccccacagttcggactggggtctgcaacccgaccccacgaagctggattcgctagtaatcgcgcatcagccatggcgcggtgaatacgttcccgggccttgtacacaccgcccgtcaagccatgaaagccgggggtgcctgaagtccgtgaccgcaagggacggcctagggcaaaactggtaattggggctaagtcgtaacaaggtagcc

SEQ ID NO: 9 - DNA, 1492 bp, Prevotella sp.
agagtttgatcctggctcaggatgaacgctagctacaggcttaacacatgcaagtcgaggggtaacgacagcgaaagcttgcttttgctgggcgacgaccggcgaatgggtgagtaacgcgtatccaacctgccgcaaagtagggcacagccttgcgaaagtaagattaatgccctatgtgctgtgatgatgacatcagaattgcagtaaaggttcaccgctttgcgatggggatgcgtctgattaggttgttggcggggtaacggcccaccaagcccgcgatcagtaggggttctgagaggaaggtcccccacattggaactgagacacggtccaaactcctacgggaggcagcagtgaggaatattggtcaatgggcgagagcctgaaccagccaagtagcgtgcgggacgaaggccctatgggttgtaaaccgcttttacggggggataaagtgagtgacgtgtcattcattgcaggtaccccgcgaataaggaccggctaattccgtgccagcagccgcggtaatacggaaggtccgggcgttatccggatttattgggtttaaagggagcacaggccggctgtcaagcgtgttgtgaaatgtaggcgctcaacgcctgacttgcagcgcgaactgacggtcttgagtgcgcgcaacgttggcggaatttgtcgtgtagcggtgaaatgcttagatatgacgaagaactccgattgcgaaggcagctgacgggagcgttactgacgcttaagctcgaaagcgcgggtatcgaacaggattagataccctggtagtccgcgcggtaaacgatggatgcccgctgtttgcgtctaacgtaagcggccaagtgaaaacgttaagcatcccacctggggagtacgccggcaacggtgaaactcaaaggaattgacgggggcccgcacaagcggaggaacatgtggtttaattcgatgatacgcgaggaaccttacccgggcttgaattgctgaggaaagatccagagatggtgatgcccttcggggcctcagtgaaggtgctgcatggttgtcgtcagctcgtgccgtgaggtgtcggcttaagtgccataacgagcgcaacccctctcttcagttgccatcaggctatgctgggcactctggagacactgccaccgcaaggtgtgaggaaggtggggatgacgtcaaatcagcacagcccttacgtccggggctacacacgtgttacaatagggggcacagagagccgggtgcgcgcaagcttgcccaaatccttaaatccccccacagttcggactggggtctgcaacccgaccccacgaagctggattcgctagtaatcgcgcatcagccatggcgcggtgaatacgttcccgggccttgtacacaccgcccgtcaagccatgaaagccgggggtgcctgaagtccgtgaccgcaagggacggcctagggcaaaactggtaattggggctaagtcgtaacaaggtagcc

SEQ ID NO: 10 - DNA, 1491 bp, Prevotella sp.
agagtttgatcatggctcaggatgaacgctagctacaggcttaacacatgcaagtcgaggggtaacgacagcgaaagcttgcttttgctgggcgacgaccggcgaatgggtgagtaacgcgtatccaacctgccgcaaagtagggcgcagccttgcgaaagtaagattaatgccctatgtgctgtgatgatgacatcagaattgcagtaaaggttcaccgctttgcgatggggatgcgtctgattaggttgttggcggggtaacggtccaccaagcccgcgatcagtaggggttctgagaggaaggtcccccacattggaactgagacacagtccaaactcctacgggaggcagcagtgaggaatattggtcaatgggcgagagcctgaaccagccaagtagcgtgcgggacgaaggccctatgggttgtaaaccgcttttacgggggataaagtgagtgacgtgtcattcattgcaggtaccccgcgaataaggaccggctaattccgtgccagcagccgcggtaatacggaaggtccgggcgttatccggatttattgggtttaaagggagcacaggccggctgtcaagcgtgttgtgaaatgtaggcgctcaacgcctgacttgcagcgcgaactgacggtcttgagtgcgcgcaacgttggcggaatttgtcgtgtagcggtgaaatgcttagatatgacgaagaactccgattgcgaaggcagctgacgtgagcgttactgacgcttaagctcgaaagcgcgggtatcgaacaggattagataccctggtagtccgcgcggtaaacgatggatgcccgctgtttgcgtctaacgtaagcggccaagtgaaaacgttaagcatcccacctggggagtacgccggcaacggtgaaactcaaaggaattgacgggggcccgcacaagcggaggaacatgtggtttaattcgatgatacgcgaggaaccttacccgggcttgaattgctgaggaaagatccagagatggtgatgcccttcggggcctcagtgaaggtgctgcatggttgtcgtcagctcgtgccgtgaggtgtcggcttaagtgccataacgagcgcaacccctctcttcagttgccatcaggctatgctgggcactctggagacactgccaccgcaaggtgtgaggaaggtggggatgacgtcaaatcagcacggcccttacgtccggggctacacacgtgttacaatggggggcacagagagtcgggtgcgcgcaagcttgcccaaatccttaaatccccccacagttcggactggggtctgcaacccgaccccacgaagctggattcgctagtaatcgcgcatcagccatggcgcggtgaatacgttcccgggccttgtacacaccgcccgtcaagccatgaaagccgggggtgcctgaagtccgtgaccgcaagggacggcctagggcaaaactggtaattggggctaagtcgtaacaaggtagcc

SEQ ID NO: 11 - DNA, 1492 bp, Prevotella sp.
agagtttgatcctggctcaggatgaacgctagctacaggcttaacacatgcaagtcgaggggtaacgacagcgaaagcttgcttttgctgggcgacgaccggcgaatgggtgagtaacgcgtatccaacctgccgcaaagtagggcacagccttgcgaaagtaagattaatgccctatgtgctgtgatgaggacatctgaattgcagtaaaggttcaccgctttgcgatggggatgcgtctgattaggttgttggcggggtaacggcccaccaagcccgcgatcagtaggggttctgagaggaaggtcccccacattggaactgagacacggtccaaactcctacgggaggcagcagtgaggaatattggtcaatgggcgagagcctgaaccagccaagtagcgtgcgggacgaaggccctatgggttgtaaaccgcttttacggggggataaagtgcgtgacgtgtcattcattgcaggtaccccgcgaataaggaccggctaattccgtgccagcagccgcggtaatacggaaggtccgggcgttatccggatttattgggtttaaagggagcacaggccggctgtcaagcgtgttgtgaaatgtaggtgctcaacgcctgacttgcagcgcgaactgacggtcttgagtgcgcgcaacgttggcggaatttgtcgtgtagcggtgaaatgcttagatatgacgaagaactccgattgcgaaggcagctgacgggagcgttactgacgcttaagctcgaaagcgcgggtatcgaacaggattagataccctggtagtccgcgcggtaaacgatggatgcccgctgtttgcgtctaacgtaagcggccaagtgaaaacgttaagcatcccacctggggagtacgccggcaacggtgaaactcaaaggaattgacgggggcccgcacaagcggaggaacatgtggtttaattcgatgatacgcgaggaaccttacccgggcttgaattgctgaggaaagatccagagatggtgatgcccttcggggcctcagtgaaggtgctgcatggttgtcgtcagctcgtgccgtgaggtgtcggcttaagtgccataacgagcgcaacccctctcttcagttgccatcaggctatgctgggcactctggagacactgccaccgcaaggtgtgaggaaggtggggatgacgtcaaatcagcacggcccttacgtccggggctacacacgtgttacaatggggggcacagagagccgggtgcgcgcaagcttgcccaaatccttaaatccccccacagttcggactggggtctgcaacccgaccccacgaagctggattcgctagtaatcgcgcatcagccatggcgcggtgaatacgttcccgggccttgtacacaccgcccgtcaagccatgaaagccgggggtgcctgaagtccgtgaccgcaagggacggcctagggcaaaactggtaattggggctaagtcgtaacaaggtagcc

SEQ ID NO: 12 - DNA, 20 bp, Artificial Sequence
  primer
agagtttgatcmtggctcag

SEQ ID NO: 13 - DNA, 19 bp, Artificial Sequence
  primer
ggytaccttgttacgactt